European Patent Application EP 4 613 778 A2, published September 10, 2025. Title: Anti-complement C1s antibodies and uses thereof. Applicant: Bioverativ USA Inc. Application WO PCT/EP2013/066783, filed October 25, 2013. The sequence listing filed with the application follows.

SEQUENCE LISTING (159 sequences)

SEQ ID NO: 1 - protein, 12 aa, synthetic construct
  REGION 1..12: note = Synthetic amino acid sequence
QSVDYDGDSYMN

SEQ ID NO: 2 - protein, 10 aa, synthetic construct
  REGION 1..10: note = Synthetic amino acid sequence
AASNLESGIP

SEQ ID NO: 3 - protein, 9 aa, synthetic construct
  REGION 1..9: note = Synthetic amino acid sequence
QQSNEDPWT

SEQ ID NO: 4 - protein, 12 aa, synthetic construct
  REGION 1..12: note = Synthetic amino acid sequence
GFNIKDDYIHWV

SEQ ID NO: 5 - protein, 10 aa, synthetic construct
  REGION 1..10: note = Synthetic amino acid sequence
IDPADDHTKY

SEQ ID NO: 6 - protein, 12 aa, synthetic construct
  REGION 1..12: note = Synthetic amino acid sequence
AIYGSGWAWFPY

SEQ ID NO: 7 - protein, 111 aa, synthetic construct
  REGION 1..111: note = Synthetic amino acid sequence
DIVLTQSTDYLAVSLGQRATISCKASQSVDYDGDSYMNWYQQKPGQPPKLLIYAASNLESGIPARFSGSGSGTDFTLNIHPVEEEDAATYYCQQSNEDPWTFGGGTKLEIK

SEQ ID NO: 8 - protein, 119 aa, synthetic construct
  REGION 1..119: note = Synthetic amino acid sequence
EVQLQQSGAELVRPGASVKLSCTASGFNIKDDYIHWVKQRPEQGLEWIGRIDPADDHTKYAPKFQDKATMTADTSSNTACLQLNSLTSEDTAVYYCAIYGSGWAWFPYWGQGTLVSVSA

SEQ ID NO: 9 - protein, 12 aa, synthetic construct
  REGION 1..12: note = Synthetic amino acid sequence
QSVDYDGDSYMN

SEQ ID NO: 10 - protein, 10 aa, synthetic construct
  REGION 1..10: note = Synthetic amino acid sequence
DASNLESGIP

SEQ ID NO: 11 - protein, 9 aa, synthetic construct
  REGION 1..9: note = Synthetic amino acid sequence
QQSNEDPWT

SEQ ID NO: 12 - protein, 12 aa, synthetic construct
  REGION 1..12: note = Synthetic amino acid sequence
GFNIKDDYIHWV

SEQ ID NO: 13 - protein, 10 aa, synthetic construct
  REGION 1..10: note = Synthetic amino acid sequence
IDPADGHTKY

SEQ ID NO: 14 - protein, 12 aa, synthetic construct
  REGION 1..12: note = Synthetic amino acid sequence
ARYGYGREVFDY

SEQ ID NO: 15 - protein, 111 aa, synthetic construct
  REGION 1..111: note = Synthetic amino acid sequence
DIVLTQSPASLAVSLGQRATISCKASQSVDYDGDSYMNWYQQKTGQPPKILIYDASNLESGIPARFSGSGSGTDFTLNIHPVEEEDAAIYYCQQSNEDPWTFGGGTKLEIK

SEQ ID NO: 16 - protein, 119 aa, synthetic construct
  REGION 1..119: note = Synthetic amino acid sequence
EVKLQQSGAELVRPGASVKLSCTASGFNIKDDYIHWVKQRPEQGLEWIGRIDPADGHTKYAPKFQVKATITADTSSNTAYLQLSSLTSEDTAVYYCARYGYGREVFDYWGQGTTLTVSS

SEQ ID NO: 17 - protein, 12 aa, synthetic construct
  REGION 1..12: note = Synthetic amino acid sequence
SSISYMHWYHQK

SEQ ID NO: 18 - protein, 10 aa, synthetic construct
  REGION 1..10: note = Synthetic amino acid sequence
DTSKLASGVP

SEQ ID NO: 19 - protein, 8 aa, synthetic construct
  REGION 1..8: note = Synthetic amino acid sequence
HQRSSFPT

SEQ ID NO: 20 - protein, 12 aa, synthetic construct
  REGION 1..12: note = Synthetic amino acid sequence
GYTFTRYWMHWV

SEQ ID NO: 21 - protein, 10 aa, synthetic construct
  REGION 1..10: note = Synthetic amino acid sequence
INPSNSDTDY

SEQ ID NO: 22 - protein, 12 aa, synthetic construct
  REGION 1..12: note = Synthetic amino acid sequence
TIDDSVYGWFAY

SEQ ID NO: 23 - protein, 105 aa, synthetic construct
  REGION 1..105: note = Synthetic amino acid sequence
DIVITQSPAIMSASPGERVTMTCSASSSISYMHWYHQKPGTSPKRWIYDTSKLASGVPARFSGSGSGTSYSLTISSMEAEDAATYYCHQRSSFPTFGAGTKLELK

SEQ ID NO: 24 - protein, 119 aa, synthetic construct
  REGION 1..119: note = Synthetic amino acid sequence
QVQLQQPGAELVRPGASVKLSCKVSGYTFTRYWMHWVKQRPGQGLEWIGEINPSNSDTDYNEEFKSKATLTVDKSSSTAYMHLSSLTSEDSAVYYCTIDDSVYGWFAYWGQGTLVTVSA

SEQ ID NO: 25 - protein, 12 aa, synthetic construct
  REGION 1..12: note = Synthetic amino acid sequence
QSVDYDGDSYMN

SEQ ID NO: 26 - protein, 10 aa, synthetic construct
  REGION 1..10: note = Synthetic amino acid sequence
AASNLEFGIP

SEQ ID NO: 27 - protein, 9 aa, synthetic construct
  REGION 1..9: note = Synthetic amino acid sequence
QQSNEDPWT

SEQ ID NO: 28 - protein, 12 aa, synthetic construct
  REGION 1..12: note = Synthetic amino acid sequence
GFNIKDDYIHWV

SEQ ID NO: 29 - protein, 10 aa, synthetic construct
  REGION 1..10: note = Synthetic amino acid sequence
IDPADDHTKY

SEQ ID NO: 30 - protein, 12 aa, synthetic construct
  REGION 1..12: note = Synthetic amino acid sequence
AIYGSGWAWFPY

SEQ ID NO: 31 - protein, 111 aa, synthetic construct
  REGION 1..111: note = Synthetic amino acid sequence
DIVMTQSPDYLAVSLGQRAPISCKASQSVDYDGDSYMNWYQQKPGQPPKLLIYAASNLEFGIPTRFSGSGFGTDFPLNIHPVEEEDAATYYCQQSNEDPWTFGGGPKLEIK

SEQ ID NO: 32 - protein, 149 aa, synthetic construct
  REGION 1..149: note = Synthetic amino acid sequence
QVQLQQSGAELVRPGASVKLSCTASGFNIKDDYIHWVKQRPEQGLEWIGRIDPADDHTKYAPKFQDKATMTADTSSNTACLQLNSLTSEDTAVYYCAIYGSGWAWFPYWGQGTLVSVSAAKTTAPSVYPLAPVCGDTTGSSVTLGCLVK

SEQ ID NO: 33 - protein, 12 aa, synthetic construct
  REGION 1..12: note = Synthetic amino acid sequence
QSVDYDGDSYMN

SEQ ID NO: 34 - protein, 10 aa, synthetic construct
  REGION 1..10: note = Synthetic amino acid sequence
DASNLEFGIP

SEQ ID NO: 35 - protein, 9 aa, synthetic construct
  REGION 1..9: note = Synthetic amino acid sequence
QQSNEDPWT

SEQ ID NO: 36 - protein, 12 aa, synthetic construct
  REGION 1..12: note = Synthetic amino acid sequence
GFNIKDDYIHWV

SEQ ID NO: 37 - protein, 10 aa, synthetic construct
  REGION 1..10: note = Synthetic amino acid sequence
IDPADGHTKY

SEQ ID NO: 38 - protein, 12 aa, synthetic construct
  REGION 1..12: note = Synthetic amino acid sequence
ARYGYGREVFDY

SEQ ID NO: 39 - protein, 111 aa, synthetic construct
  REGION 1..111: note = Synthetic amino acid sequence
DIVLTQFPTFLAVFLGQRAPISCKASQSVDYDGDSYMNWFQQKTGQPPKILIYDASNLEFGIPTRFSGSGFGTDFPLNIHPVEEEDAAIYFCQQSNEDPWTFGGGPKLEIK

SEQ ID NO: 40 - protein, 119 aa, synthetic construct; identical to SEQ ID NO: 16
  REGION 1..119: note = Synthetic amino acid sequence

SEQ ID NO: 41 - protein, 12 aa, synthetic construct
  REGION 1..12: note = Synthetic amino acid sequence
QSVDYDGDSYMN

SEQ ID NO: 42 - protein, 10 aa, synthetic construct
  REGION 1..10: note = Synthetic amino acid sequence
AASNLESGIP

SEQ ID NO: 43 - protein, 9 aa, synthetic construct
  REGION 1..9: note = Synthetic amino acid sequence
QQSNEDPWT

SEQ ID NO: 44 - protein, 12 aa, synthetic construct
  REGION 1..12: note = Synthetic amino acid sequence
GFNIKDDYIHWV

SEQ ID NO: 45 - protein, 10 aa, synthetic construct
  REGION 1..10: note = Synthetic amino acid sequence
IDPADDHTKY

SEQ ID NO: 46 - protein, 12 aa, synthetic construct
  REGION 1..12: note = Synthetic amino acid sequence
AIYGSGWAWFPY

SEQ ID NO: 47 - protein, 112 aa, synthetic construct
  REGION 1..112: note = Synthetic amino acid sequence
EFALMTQSTDYLAVSLGQRATISCKASQSVDYDGDSYMNWYQQKPGQPPKLLIYAASNLESGIPTRFSGSGFGTDFTLNIHPVEEEDAATYYCQQSNEDPWTFGGGPKLEIK

SEQ ID NO: 48 - protein, 119 aa, synthetic construct
  REGION 1..119: note = Synthetic amino acid sequence
EVKLEQSGAELVRPGASVKLSCTASGFNIKDDYIHWVKQRPEQGLEWIGRIDPADDHTKYAPKFQDKATMTADTSSNTACLQLNSLTSEDTAVYYCAIYGSGWAWFPYWGQGTLVSVSA

SEQ ID NO: 49 - protein, 12 aa, synthetic construct
  REGION 1..12: note = Synthetic amino acid sequence
SSISYMYWFQQK

SEQ ID NO: 50 - protein, 10 aa, synthetic construct
  REGION 1..10: note = Synthetic amino acid sequence
DTSKLASGVP

SEQ ID NO: 51 - protein, 8 aa, synthetic construct
  REGION 1..8: note = Synthetic amino acid sequence
HQRSSDPT

SEQ ID NO: 52 - protein, 12 aa, synthetic construct
  REGION 1..12: note = Synthetic amino acid sequence
GYSFTGYYIHWV

SEQ ID NO: 53 - protein, 10 aa, synthetic construct
  REGION 1..10: note = Synthetic amino acid sequence
INPTTNDTTY

SEQ ID NO: 54 - protein, 12 aa, synthetic construct
  REGION 1..12: note = Synthetic amino acid sequence
SRDISGPAWFAY

SEQ ID NO: 55 - protein, 106 aa, synthetic construct
  REGION 1..106: note = Synthetic amino acid sequence
DIVLTQTTAIMSASPGEKVTMTCSASSSISYMYWFQQKPGTSPKRWIYDTSKLASGVPARFSGSGSGTSYSLTISTMEAEDAATYYCHQRSSDPTFGGGTKLEINR

SEQ ID NO: 56 - protein, 119 aa, synthetic construct
  REGION 1..119: note = Synthetic amino acid sequence
EVQLQQSGPELVKPGASVKISCKASGYSFTGYYIHWVKQSPEKSLEWIGEINPTTNDTTYNQKFKAKATLTVDKSSNTAYMQLKSLTSEDSAVYYCSRDISGPAWFAYWGQGTLVTVSA

SEQ ID NO: 57 - protein, 5 aa, synthetic construct
  REGION 1..5: note = Synthetic amino acid sequence
SSISY

SEQ ID NO: 58 - protein, 10 aa, synthetic construct
  REGION 1..10: note = Synthetic amino acid sequence
DTSKLASGVP

SEQ ID NO: 59 - protein, 8 aa, synthetic construct
  REGION 1..8: note = Synthetic amino acid sequence
HQRSSFPP

SEQ ID NO: 60 - protein, 12 aa, synthetic construct
  REGION 1..12: note = Synthetic amino acid sequence
GYTFTRYWMHWV

SEQ ID NO: 61 - protein, 10 aa, synthetic construct
  REGION 1..10: note = Synthetic amino acid sequence
INPSNSDTDY

SEQ ID NO: 62 - protein, 12 aa, synthetic construct
  REGION 1..12: note = Synthetic amino acid sequence
TIDDSVYGWFAY

SEQ ID NO: 63 - protein, 105 aa, synthetic construct
  REGION 1..105: note = Synthetic amino acid sequence
DIVMTQSPAIMFASPGERVTMTCSASSSISYMPWYPQKPGPSPKRWIYDTSKLASGVPARFSGSGFGTFYSLTISSMEAEDAAPYYCHQRSSFPPFGAGTKLELK

SEQ ID NO: 64 - protein, 119 aa, synthetic construct; identical to SEQ ID NO: 24
  REGION 1..119: note = Synthetic amino acid sequence

SEQ ID NO: 65 - protein, 12 aa, synthetic construct
  REGION 1..12: note = Synthetic amino acid sequence
SSISYMHWYQQK

SEQ ID NO: 66 - protein, 10 aa, synthetic construct
  REGION 1..10: note = Synthetic amino acid sequence
DTSKLASGVP

SEQ ID NO: 67 - protein, 8 aa, synthetic construct
  REGION 1..8: note = Synthetic amino acid sequence
HQRSFYLT

SEQ ID NO: 68 - protein, 12 aa, synthetic construct
  REGION 1..12: note = Synthetic amino acid sequence
GYTFTDYAMHCV

SEQ ID NO: 69 - protein, 10 aa, synthetic construct
  REGION 1..10: note = Synthetic amino acid sequence
ISIYNGDASY

SEQ ID NO: 70 - protein, 17 aa, synthetic construct
  REGION 1..17: note = Synthetic amino acid sequence
VREAPYLITTVFYAMDY

SEQ ID NO: 71 - protein, 105 aa, synthetic construct
  REGION 1..105: note = Synthetic amino acid sequence
DIVMTQSPAIMSASPGEKVTMTCSANSSISYMHWYQQKPGTSPKRWIYDTSKLASGVPTRFSGSGSGTSYSLTISSMEAEDAATYYCHQRSFYLTFGSGTKLEIK

SEQ ID NO: 72 - protein, 124 aa, synthetic construct
  REGION 1..124: note = Synthetic amino acid sequence
EVKLQQSGAELVRPGVSVKISCKVSGYTFTDYAMHCVKQSHAKSLEWIGVISIYNGDASYNQKFKDKATMTVDKSSSTSYMDLARLTSEESAVYNCVREAPYLITTVFYAMDYWGQGTSVTVSS

SEQ ID NO: 73 - protein, 12 aa, synthetic construct
  REGION 1..12: note = Synthetic amino acid sequence
SSISYMHWYHQK

SEQ ID NO: 74 - protein, 10 aa, synthetic construct
  REGION 1..10: note = Synthetic amino acid sequence
DTSKLASGVP

SEQ ID NO: 75 - protein, 8 aa, synthetic construct
  REGION 1..8: note = Synthetic amino acid sequence
HQRSSFPT

SEQ ID NO: 76 - protein, 12 aa, synthetic construct
  REGION 1..12: note = Synthetic amino acid sequence
GYTFTRYWMHWV

SEQ ID NO: 77 - protein, 10 aa, synthetic construct
  REGION 1..10: note = Synthetic amino acid sequence
INPSNSDTDY

SEQ ID NO: 78 - protein, 12 aa, synthetic construct
  REGION 1..12: note = Synthetic amino acid sequence
TIDDSAYGWFAY

SEQ ID NO: 79 - protein, 105 aa, synthetic construct
  REGION 1..105: note = Synthetic amino acid sequence
DIVLTQSTAIMSASPGERVTMTCSASSSISYMHWYHQKPGTSPKRWIYDTSKLASGVPARFSGSGSGTSYSLAISSMEAEDAATYYCHQRSSFPTFGAGTKLELK

SEQ ID NO: 80 - protein, 119 aa, synthetic construct
  REGION 1..119: note = Synthetic amino acid sequence
QVQLQQSGAELVRPGASVKLSCKVSGYTFTRYWMHWVKQRPGQGLEWIGEINPSNSDTDYNEEFKSKATLTVDKSSSTAYMHLSNLTSEDSAVYYCTIDDSAYGWFAYWGQGTLVTVSA

SEQ ID NO: 81 - protein, 12 aa, synthetic construct
  REGION 1..12: note = Synthetic amino acid sequence
QSVDYDGDSYMN

SEQ ID NO: 82 - protein, 10 aa, synthetic construct
  REGION 1..10: note = Synthetic amino acid sequence
AASNLESGIP

SEQ ID NO: 83 - protein, 9 aa, synthetic construct
  REGION 1..9: note = Synthetic amino acid sequence
QQSNEDPWT

SEQ ID NO: 84 - protein, 12 aa, synthetic construct
  REGION 1..12: note = Synthetic amino acid sequence
GFNIKDDYIHWV

SEQ ID NO: 85 - protein, 10 aa, synthetic construct
  REGION 1..10: note = Synthetic amino acid sequence
IDPADDHTKY

SEQ ID NO: 86 - protein, 12 aa, synthetic construct
  REGION 1..12: note = Synthetic amino acid sequence
AIYGSGWAWFPY

SEQ ID NO: 87 - protein, 111 aa, synthetic construct
  REGION 1..111: note = Synthetic amino acid sequence
DIVLTQTPDYLAVSLGQRATISCKASQSVDYDGDSYMNWYQQKPGQPPKLLIYAASNLESGIPARFSGSGSGTDFTLNIHPVEEEDAATYYCQQSNEDPWTFGGGTKLEIK

SEQ ID NO: 88 - protein, 119 aa, synthetic construct; identical to SEQ ID NO: 8
  REGION 1..119: note = Synthetic amino acid sequence

SEQ ID NO: 89 - protein, 12 aa, synthetic construct
  REGION 1..12: note = Synthetic amino acid sequence
SSISYIHWYQQK

SEQ ID NO: 90 - protein, 10 aa, synthetic construct
  REGION 1..10: note = Synthetic amino acid sequence
DTSKLASGVP

SEQ ID NO: 91 - protein, 8 aa, synthetic construct
  REGION 1..8: note = Synthetic amino acid sequence
HQRSSYLT

SEQ ID NO: 92 - protein, 12 aa, synthetic construct
  REGION 1..12: note = Synthetic amino acid sequence
GYSFTGFYMQWV

SEQ ID NO: 93 - protein, 10 aa, synthetic construct
  REGION 1..10: note = Synthetic amino acid sequence
INPTTGDETY

SEQ ID NO: 94 - protein, 14 aa, synthetic construct
  REGION 1..14: note = Synthetic amino acid sequence
ASDFYDGSFAWFEY

SEQ ID NO: 95 - protein, 105 aa, synthetic construct
  REGION 1..105: note = Synthetic amino acid sequence
DIVLTQSPVIMSASPGEKVTMTCSASSSISYIHWYQQKPGTSPKRWIYDTSKLASGVPARFSGSGSGTSYSLTISSMEAEDAATYYCHQRSSYLTFGSGTKLEIK

SEQ ID NO: 96 - protein, 120 aa, synthetic construct
  REGION 1..120: note = Synthetic amino acid sequence
EVQLQQSGPELVKPGASVKISCKASGYSFTGFYMQWVKQSPEKNLEWIGEINPTTGDETYNQKFQAKATLTVDKSSSTAYMQLKSLTSEDSAVYFCASDFYDGSFAWFEYWGKDYLTVSA

SEQ ID NO: 97 - protein, 12 aa, synthetic construct
  REGION 1..12: note = Synthetic amino acid sequence
SSINYMHWYQQK

SEQ ID NO: 98 - protein, 10 aa, synthetic construct
  REGION 1..10: note = Synthetic amino acid sequence
DTSKLASGVP

SEQ ID NO: 99 - protein, 8 aa, synthetic construct
  REGION 1..8: note = Synthetic amino acid sequence
HQRSDSLT

SEQ ID NO: 100 - protein, 12 aa, synthetic construct
  REGION 1..12: note = Synthetic amino acid sequence
GYSFTGYYMHWV

SEQ ID NO: 101 - protein, 10 aa, synthetic construct
  REGION 1..10: note = Synthetic amino acid sequence
INPSIGDITY

SEQ ID NO: 102 - protein, 14 aa, synthetic construct
  REGION 1..14: note = Synthetic amino acid sequence
ASDYYGGGFAWFAY

SEQ ID NO: 103 - protein, 105 aa, synthetic construct
  REGION 1..105: note = Synthetic amino acid sequence
DIVMTQSPAIMSASSGEKVTMTCSASSSINYMHWYQQKPGTSPKRWIYDTSKLASGVPARFSGSGSGTSYSLTISSMEAEDTATYYCHQRSDSLTFGSGTKLEIK

SEQ ID NO: 104 - protein, 121 aa, synthetic construct
  REGION 1..121: note = Synthetic amino acid sequence
QVKLQQSGPELVKPGTSVRISCKTSGYSFTGYYMHWVKQSPEKSLEWIGEINPSIGDITYNQRFKAKATLTVDKSSSTAYMQLKSLTSEDSAVYYCASDYYGGGFAWFAYWGQGTLVTVSA

SEQ ID NO: 105 - protein, 12 aa, synthetic construct
  REGION 1..12: note = Synthetic amino acid sequence
SSISYMHWYHQK

SEQ ID NO: 106 - protein, 10 aa, synthetic construct
  REGION 1..10: note = Synthetic amino acid sequence
DTSKLASGVP

SEQ ID NO: 107 - protein, 8 aa, synthetic construct
  REGION 1..8: note = Synthetic amino acid sequence
HQRSSFPT

SEQ ID NO: 108 - protein, 12 aa, synthetic construct
  REGION 1..12: note = Synthetic amino acid sequence
GYTFTRYWMHWV

SEQ ID NO: 109 - protein, 10 aa, synthetic construct
  REGION 1..10: note = Synthetic amino acid sequence
INPSNSDTDY

SEQ ID NO: 110 - protein, 12 aa, synthetic construct
  REGION 1..12: note = Synthetic amino acid sequence
TIDDSAYGWFAY

SEQ ID NO: 111 - protein, 105 aa, synthetic construct
  REGION 1..105: note = Synthetic amino acid sequence
DIVMTQSPAIMSASPGERVTMTCSASSSISYMHWYHQKPGTSPKRWIYDTSKLASGVPARFSGSGSGTSYSLTISSMEAEDAATYYCHQRSSFPTFGAGTKLELK

SEQ ID NO: 112 - protein, 119 aa, synthetic construct
  REGION 1..119: note = Synthetic amino acid sequence
QVQLQQPGAELVRPGASVKLSCKVSGYTFTRYWMHWVKQRPGQGLEWIGEINPSNSDTDYNEEFKSKATLTVDKSSSTAYMHLSSLTSEDSAVYYCTIDDSAYGWFAYWGQGTLVTVSA

SEQ ID NO: 113 - protein, 673 aa, Homo Sapiens
EPTMYGEILSPNYPQAYPSEVEKSWDIEVPEGYGIHLYFTHLDIELSENCAYDSVQIISGDTEEGRLCGQRSSNNPHSPIVEEFQVPYNKLQVIFKSDFSNEERFTGFAAYYVATDINECTDFVDVPCSHFCNNFIGGYFCSCPPEYFLHDDMKNCGVNCSGDVFTALIGEIASPNYPKPYPENSRCEYQIRLEKGFQVVVTLRREDFDVEAADSAGNCLDSLVFVAGDRQFGPYCGHGFPGPLNIETKSNALDIIFQTDLTGQKKGWKLRYHGDPMPCPKEDTPNSVWEPAKAKYVFRDVVQITCLDGFEVVEGRVGATSFYSTCQSNGKWSNSKLKCQPVDCGIPESIENGKVEDPESTLFGSVIRYTCEEPYYYMENGGGGEYHCAGNGSWVNEVLGPELPKCVPVCGVPREPFEEKQRIIGGSDADIKNFPWQVFFDNPWAGGALINEYWVLTAAHVVEGNREPTMYVGSTSVQTSRLAKSKMLTPEHVFIHPGWKLLEVPEGRTNFDNDIALVRLKDPVKMGPTVSPICLPGTSSDYNLMDGDLGLISGWGRTEKRDRAVRLKAARLPVAPLRKCKEVKVEKPTADAEAYVFTPNMICAGGEKGMDSCKGDSGGAFAVQDPNDKTKFYAAGLVSWGPQCGTYGLYTRVKNYVDWIMKTMQENSTPRED

SEQ ID NO: 114 - protein, 5 aa, synthetic construct
  REGION 1..5: note = Synthetic amino acid sequence
GSGGS

SEQ ID NO: 115 - protein, 4 aa, synthetic construct
  REGION 1..4: note = Synthetic amino acid sequence
GGGS

SEQ ID NO: 116 - protein, 4 aa, synthetic construct
  REGION 1..4: note = Synthetic amino acid sequence
GGSG

SEQ ID NO: 117 - protein, 5 aa, synthetic construct
  REGION 1..5: note = Synthetic amino acid sequence
GGSGG

SEQ ID NO: 118 - protein, 5 aa, synthetic construct
  REGION 1..5: note = Synthetic amino acid sequence
GSGSG

SEQ ID NO: 119 - protein, 5 aa, synthetic construct
  REGION 1..5: note = Synthetic amino acid sequence
GSGGG

SEQ ID NO: 120 - protein, 5 aa, synthetic construct
  REGION 1..5: note = Synthetic amino acid sequence
GGGSG

SEQ ID NO: 121 - protein, 5 aa, synthetic construct
  REGION 1..5: note = Synthetic amino acid sequence
GSSSG

SEQ ID NO: 122 - protein, 9 aa, synthetic construct
  REGION 1..9: note = Synthetic amino acid sequence
YPYDVPDYA

SEQ ID NO: 123 - protein, 8 aa, synthetic construct
  REGION 1..8: note = Synthetic amino acid sequence
DYKDDDDK

SEQ ID NO: 124 - protein, 10 aa, synthetic construct
  REGION 1..10: note = Synthetic amino acid sequence
EQKLISEEDL

SEQ ID NO: 125 - protein, 5 aa, synthetic construct
  REGION 1..5: note = Synthetic amino acid sequence
HHHHH

SEQ ID NO: 126 - protein, 6 aa, synthetic construct
  REGION 1..6: note = Synthetic amino acid sequence
HHHHHH

SEQ ID NO: 127 - protein, 8 aa, synthetic construct
  REGION 1..8: note = Synthetic amino acid sequence
WSHPQFEK

SEQ ID NO: 128 - protein, 5 aa, synthetic construct
  REGION 1..5: note = Synthetic amino acid sequence
RYIRS

SEQ ID NO: 129 - protein, 4 aa, synthetic construct
  REGION 1..4: note = Synthetic amino acid sequence
FHHT

SEQ ID NO: 130 - protein, 17 aa, synthetic construct
  REGION 1..17: note = Synthetic amino acid sequence
WEAAAREACCRECCARA

SEQ ID NO: 131 - protein, 19 aa, synthetic construct
  REGION 1..19: note = Synthetic amino acid sequence
TFFYGGCRGKRNNFKTEEY

SEQ ID NO: 132 - protein, 19 aa, synthetic construct
  REGION 1..19: note = Synthetic amino acid sequence
TFFYGGSRGKRNNFKTEEY

SEQ ID NO: 133 - protein, 20 aa, synthetic construct
  REGION 1..20: note = Synthetic amino acid sequence
CTFFYGGSRGKRNNFKTEEY

SEQ ID NO: 134 - protein, 20 aa, synthetic construct
  REGION 1..20: note = Synthetic amino acid sequence
TFFYGGSRGKRNNFKTEEYC

SEQ ID NO: 135 - protein, 16 aa, synthetic construct
  REGION 1..16: note = Synthetic amino acid sequence
TFVYGGCRAKRNNFKS

SEQ ID NO: 136 - protein, 25 aa, synthetic construct [sequence omitted]

SEQ ID NO: 137 - protein, 13 aa, synthetic construct
  REGION 1..13: note = Synthetic peptide
WVRQAPGKGLEWV

SEQ ID NO: 138 - protein, 30 aa, synthetic construct
  REGION 1..30: note = Synthetic peptide
RFTISRDNSKNTLYLQMNSLRAEDTAVYYC

SEQ ID NO: 139 - protein, 11 aa, synthetic construct
  REGION 1..11: note = Synthetic peptide
WGQGTLVTVSS

SEQ ID NO: 140 - protein, 30 aa, synthetic construct
  REGION 1..30: note = Synthetic peptide
RFTISADTSKNTAYLQMNSLRAEDTAVYYC

SEQ ID NO: 141 - protein, 25 aa, synthetic construct [sequence omitted]

SEQ ID NO: 142 - protein, 13 aa, synthetic construct
  REGION 1..13: note = Synthetic peptide
WVRQAPGQGLEWM

SEQ ID NO: 143 - protein, 30 aa, synthetic construct
  REGION 1..30: note = Synthetic peptide
RVTITADTSTSTAYMELSSLRSEDTAVYYC

SEQ ID NO: 144 - protein, 25 aa, synthetic construct
  REGION 1..25: note = Synthetic peptide
QVQLQESGPGLVKPSQTLSLTCTVS

SEQ ID NO: 145 - protein, 13 aa, synthetic construct
  REGION 1..13: note = Synthetic peptide
WIRQPPGKGLEWI

SEQ ID NO: 146 - protein, 30 aa, synthetic construct
  REGION 1..30: note = Synthetic peptide
RVTISVDTSKNQFSLKLSSVTAADTAVYYC

SEQ ID NO: 147 - protein, 23 aa, synthetic construct
  REGION 1..23: note = Synthetic peptide
DIQMTQSPSSLSASVGDRVTITC

SEQ ID NO: 148 - protein, 15 aa, synthetic construct
  REGION 1..15: note = Synthetic peptide
WYQQKPGKAPKLLIY

SEQ ID NO: 149 - protein, 32 aa, synthetic construct
  REGION 1..32: note = Synthetic peptide
GVPSRFSGSGSGTDFTLTISSLQPEDFATYYC

SEQ ID NO: 150 - protein, 10 aa, synthetic construct
  REGION 1..10: note = Synthetic peptide
FGQGTKVEIK

SEQ ID NO: 151 - protein, 23 aa, synthetic construct
  REGION 1..23: note = Synthetic peptide
DIVMTQSPLSLPVTPGEPASISC

SEQ ID NO: 152 - protein, 15 aa, synthetic construct
  REGION 1..15: note = Synthetic peptide
WYLQKPGQSPQLLIY

SEQ ID NO: 153 - protein, 32 aa, synthetic construct
  REGION 1..32: note = Synthetic peptide
GVPDRFSGSGSGTDFTLKISRVEAEDVGVYYC

SEQ ID NO: 154 - protein, 23 aa, synthetic construct
  REGION 1..23: note = Synthetic peptide
EIVLTQSPGTLSLSPGERATLSC

SEQ ID NO: 155 - protein, 15 aa, synthetic construct
  REGION 1..15: note = Synthetic peptide
WYQQKPGQAPRLLIY

SEQ ID NO: 156 - protein, 32 aa, synthetic construct
  REGION 1..32: note = Synthetic peptide
GIPDRFSGSGSGTDFTLTISRLEPEDFAVYYC

SEQ ID NO: 157 - protein, 23 aa, synthetic construct
  REGION 1..23: note = Synthetic peptide
DIVMTQSPDSLAVSLGERATINC

SEQ ID NO: 158 - protein, 15 aa, synthetic construct
  REGION 1..15: note = Synthetic peptide
WYQQKPGQPPKLLIY

SEQ ID NO: 159 - protein, 32 aa, synthetic construct
  REGION 1..32: note = Synthetic peptide
GVPDRFSGSGSGTDFTLTISSLQAEDFAVYYC